European Patent Application EP 4 206 674 A1, published July 5, 2023. Title: HIGH-THROUGHPUT SEROTYPING AND ANTIBODY PROFILING ASSAYS. Applicant: Encodia, Inc. Application EP. The sequence listing filed with the application follows.

SEQUENCE LISTING (50 sequences)

SEQ ID NO: 1 - protein, 7 aa, synthetic construct
  REGION 1..7: note = Peptide linker
  SITE 7: note = modified with azide
GSGSGSK

SEQ ID NO: 2 - DNA, 20 bp, synthetic construct
  source 1..20: mol_type = other DNA
  misc_feature 1..20: note = P5 primer
aatgatacggcgaccaccga

SEQ ID NO: 3 - DNA, 24 bp, synthetic construct
  source 1..24: mol_type = other DNA
  misc_feature 1..24: note = P7 primer
caagcagaagacggcatacgagat

SEQ ID NO: 4 - protein, 27 aa, synthetic construct
  REGION 1..27: note = CT epitope 1
TGTGVLTESNKKFLPFQQFGRDIAGGK

SEQ ID NO: 5 - protein, 27 aa, synthetic construct
  REGION 1..27: note = CT epitope 2
FAQVKQIYKTPPIKDFGGFNFSQIGGK

SEQ ID NO: 6 - protein, 27 aa, synthetic construct
  REGION 1..27: note = CT epitope 3
PDPSKPSKRSFIEDLLFNKVTLADGGK

SEQ ID NO: 7 - protein, 27 aa, synthetic construct
  REGION 1..27: note = CT epitope 4
YDPLQPELDSFKEELDKYFKNHTSGGK

SEQ ID NO: 8 - protein, 27 aa, synthetic construct
  REGION 1..27: note = CT epitope 5
SSSSGSSSKFDEDDSEPVLKGVKLGGK

SEQ ID NO: 9 - protein, 33 aa, synthetic construct
  REGION 1..33: note = CT epitope 6
NAAIVLQLPQGTTLPKGFYAEGSRGGSQASGGK

SEQ ID NO: 10 - protein, 33 aa, synthetic construct
  REGION 1..33: note = CT epitope 7
GDAALALLLLDRLNQLESKMSGKGQQQQGQGGK

SEQ ID NO: 11 - protein, 26 aa, synthetic construct
  REGION 1..26: note = CT epitope 8
GQQQQGQTVTKKSAAEASKKPRQGGK

SEQ ID NO: 12 - protein, 27 aa, synthetic construct
  REGION 1..27: note = CT epitope 9
DAYKTFPPTEPKKDKKKKADETQAGGK

SEQ ID NO: 13 - protein, 27 aa, synthetic construct
  REGION 1..27: note = CT epitope 10
LPQRQKKQQTVTLLPAADLDDFSKGGK

SEQ ID NO: 14 - protein, 27 aa, synthetic construct
  REGION 1..27: note = CT epitope 11
PGPRPPTRRQRHDRQRGLVWEDDDGGK

SEQ ID NO: 15 - protein, 23 aa, synthetic construct
  REGION 1..23: note = CT epitope 12
SNSESIPALTAAETGHTSQVGGK

SEQ ID NO: 16 - protein, 18 aa, synthetic construct
  REGION 1..18: note = CT epitope 13
RRPPPGRRPFFHPVAGGK

SEQ ID NO: 17 - protein, 33 aa, synthetic construct
  REGION 1..33: note = CT epitope 14
RRHTQKAPKRIRLPHIREDDQPSSHQPLFYGGK

SEQ ID NO: 18 - protein, 28 aa, synthetic construct
  REGION 1..28: note = CT epitope 15
NPIENYVDEVLNEVLVVPNINSSHPGGK

SEQ ID NO: 19 - protein, 28 aa, synthetic construct
  REGION 1..28: note = CT epitope 16
QDNSDIKVVPRRKAKIIRDYGKQMAGGK

SEQ ID NO: 20 - protein, 14 aa, synthetic construct
  REGION 1..14: note = CT epitope 17
YPYDVPDYASLGGK

SEQ ID NO: 21 - protein, 14 aa, synthetic construct
  REGION 1..14: note = CT epitope 18
YADVYPSYPDLGGK

SEQ ID NO: 22 - protein, 21 aa, synthetic construct
  REGION 1..21: note = H3N2 epitope
LGHHAVPNGTLVKTITNDGGK

SEQ ID NO: 23 - protein, 27 aa, synthetic construct
  REGION 1..27: note = H1N1 epitope
FAWRSRNENERPSLPPKQKREVAGGGK

SEQ ID NO: 24 - protein, 20 aa, synthetic construct
  REGION 1..20: note = H1N1 epitope
GKEVLVLWGIHHPSTTAGGK

SEQ ID NO: 25 - protein, 17 aa, synthetic construct
  REGION 1..17: note = H1N1 epitope
SLTSLPFQNIHPITGGK

SEQ ID NO: 26 - protein, 17 aa, synthetic construct
  REGION 1..17: note = H1N1 epitope
TASSWSYIVETSSSGGK

SEQ ID NO: 27 - protein, 23 aa, synthetic construct
  REGION 1..23: note = H1N1 epitope
QEGRMNYYWTLVEPGDKITFGGK

SEQ ID NO: 28 - protein, 18 aa, synthetic construct
  REGION 1..18: note = H1N1 epitope
SLVLVVSLGAISFWMGGK

SEQ ID NO: 29 - protein, 17 aa, synthetic construct
  REGION 1..17: note = H1N1 epitope
MESVKNGTYDYPKYGGK

SEQ ID NO: 30 - protein, 18 aa, synthetic construct
  REGION 1..18: note = H1N1 epitope
KLSKLRGVAPLHLGKGGK

SEQ ID NO: 31 - protein, 18 aa, synthetic construct
  REGION 1..18: note = H1N1 epitope
SFEFYHKSDNTSMESGGK

SEQ ID NO: 32 - protein, 18 aa, synthetic construct
  REGION 1..18: note = H1N1 epitope
VSLGAISFWMSSNGSGGK

SEQ ID NO: 33 - protein, 18 aa, synthetic construct
  REGION 1..18: note = H1N1 epitope
AISFWMSSNGSLQSRGGK

SEQ ID NO: 34 - protein, 17 aa, synthetic construct
  REGION 1..17: note = H1N1 epitope
WMSSNGSLQSRISIGGK

SEQ ID NO: 35 - DNA, 32 bp, synthetic construct
  source 1..32: mol_type = other DNA
  misc_feature 1..32: note = coding tag
  misc_feature 32: note = modified with C3 (three carbon) spacer
  misc_feature 1: note = modified with 5'-amino modifier C6 and 18 atoms hexaethylene glycol chain (iSP18)
cactcagtttccgtcatatcgaatcactcagt

SEQ ID NO: 36 - protein, 20 aa, synthetic construct
  REGION 1..20: note = SpyTag
CGSGSGSAHIVMVDAYKPTK

SEQ ID NO: 37 - protein, 241 aa, synthetic construct
  REGION 1..241: note = SpyCatcher-SnoopCatcher
VDTLSGLSSEQGQSGDMTIEEDSATHIKFSKRDEDGKELAGATMELRDSSGKTISTWISDGQVKDFYLYPGKYTFVETAAPDGYEVATAITFTVNEQGQVTVNGKATKGDAHIGGSGGGSGGGSGGSKPLRGAVFSLQKQHPDYPDIYGAIDQNGTYQNVRTGEDGKLTFKNLSDGKYRLFENSEPAGYKPVQNKPIVAFQIVNGEVRDVTSIVPQDIPATYEFTNGKHYITNEPIPPKGS

SEQ ID NO: 38 - protein, 556 aa, synthetic construct
  REGION 1..556: note = SpyCatcher-Protein A/G
VDTLSGLSSEQGQSGDMTIEEDSATHIKFSKRDEDGKELAGATMELRDSSGKTISTWISDGQVKDFYLYPGKYTFVETAAPDGYEVATAITFTVNEQGQVTVNGKATKGDAHIGGSGGGSGGGSGGSNAAQHDEAQQNAFYQVLNMPNLNADQRNGFIQSLKDDPSQSANVLGEAQKLNDSQAPKADAQQNNFNKDQQSAFYEILNMPNLNEAQRNGFIQSLKDDPSQSTNVLGEAKKLNESQAPKADNNFNKEQQNAFYEILNMPNLNEEQRNGFIQSLKDDPSQSANLLSEAKKLNESQAPKADNKFNKEQQNAFYEILHLPNLNEEQRNGFIQSLKDDPSQSANLLAEAKKLNDAQAPKADNKFNKEQQNAFYEILHLPNLTEEQRNGFIQSLKDDPSVSKEILAEAKKLNDAQAPKEEDSLEGSGSGTYKLILNGKTLKGETTTEAVDAATAEKVFKQYANDNGVDGEWTYDDATKTFTVTEKPEVIDASELTPAVTTYKLVINGKTLKGETTTKAVDAETAEKAFKQYANDNGVDGVWTYDDATKTFTVTE

SEQ ID NO: 39 - protein, 389 aa, Staphylococcus aureus
  REGION 1..389: note = Protein A
MKKKNIYSIRKLGVGIASVTLGTLLISGGVTPAANAAQHDEAQQNAFYQVLNMPNLNADQRNGFIQSLKDDPSQSANLLSEAKKLNESQAPKADNKFNKEQQNAFYEILHLPNLNEEQRNGFIQSLKDDPSQSANLLAEAKKLNDAQAPKADNKFNKEQQNAFYEILHLPNLTEEQRNGFIQSLKDDPSVSKEILAEAKKLNDAQAPKEEDNNKPGKEDGNKPGKEDNNKPGKEDNKKPGKEDNKKPGKEDNNKPGKEDGNKPGKEDNKKPGKEDNNKPGKEDGNKPGKEDGNGVHVVKPGDTVNDIAKANGTTADKIAADNKLADKNMIKPGQELVVDKKQPANHADANKAQALPETGEENPFIGTTVFGGLSLALGAALLAGRRREL

SEQ ID NO: 40 - protein, 448 aa, Streptococcus sp.
  REGION 1..448: note = Protein G
MEKEKKVKYFLRKSAFGLASVSAAFLVGSTVFAVDSPIEDTPIIRNGGELTNLLGNSETTLALRNEESATADLTAAAVADTVAAAAAENAGAAAWEAAAAADALAKAKADALKEFNKYGVSDYYKNLINNAKTVEGIKDLQAQVVESAKKARISEATDGLSDFLKSQTPAEDTVKSIELAEAKVLANRELDKYGVSDYHKNLINNAKTVEGVKELIDEILAALPKTDTYKLILNGKTLKGETTTEAVDAATAEKVFKQYANDNGVDGEWTYDDATKTFTVTEKPEVIDASELTPAVTTYKLVINGKTLKGETTTKAVDAETAEKAFKQYANDNGVDGVWTYDDATKTFTVTEMVTEVPGDAPTEPEKPEASIPLVPLTPATPIAKDDAKKDDTKKEDAKKPEAKKDDAKKAETLPTTGEGSNPFFTAAALAVMAGAGALAVASKRKED

SEQ ID NO: 41 - protein, 992 aa, Finegoldia magna
  REGION 1..992: note = Protein L
MKINKKLLMAALAGAIVVGGGANAYAAEEDNTDNNLSMDEISDAYFDYHGDVSDSVDPVEEEIDEALAKALAEAKETAKKHIDSLNHLSETAKKLAKNDIDSATTINAINDIVARADVMERKTAEKEEAEKLAAAKETAKKHIDELKHLADKTKELAKRDIDSATTINAINDIVARADVMERKTAEKEEAEKLAAAKETAKKHIDELKHLADKTKELAKRDIDSATTIDAINDIVARADVMERKLSEKETPEPEEEVTIKANLIFADGSTQNAEFKGTFAKAVSDAYAYADALKKDNGEYTVDVADKGLTLNIKFAGKKEKPEEPKEEVTIKVNLIFADGKTQTAEFKGTFEEATAKAYAYADLLAKENGEYTADLEDGGNTINIKFAGKETPETPEEPKEEVTIKVNLIFADGKIQTAEFKGTFEEATAKAYAYANLLAKENGEYTADLEDGGNTINIKFAGKETPETPEEPKEEVTIKVNLIFADGKTQTAEFKGTFEEATAEAYRYADLLAKVNGEYTADLEDGGYTINIKFAGKEQPGENPGITIDEWLLKNAKEEAIKELKEAGITSDLYFSLINKAKTVEGVEALKNEILKAHAGEETPELKDGYATYEEAEAAAKEALKNDDVNNAYEIVQGADGRYYYVLKIEVADEEEPGEDTPEVQEGYATYEEAEAAAKEALKEDKVNNAYEVVQGADGRYYYVLKIEDKEDEQPGEEPGENPGITIDEWLLKNAKEDAIKELKEAGISSDIYFDAINKAKTVEGVEALKNEILKAHAEKPGENPGITIDEWLLKNAKEAAIKELKEAGITAEYLFNLINKAKTVEGVESLKNEILKAHAEKPGENPGITIDEWLLKNAKEDAIKELKEAGITSDIYFDAINKAKTIEGVEALKNEILKAHKKDEEPGKKPGEDKKPEDKKPGEDKKPEDKKPGEDKKPEDKKPGKTDKDSPNKKKKAKLPKAGSEAEILTLAAAALSTAAGAYVSLKKRK

SEQ ID NO: 42 - protein, 12 aa, synthetic construct
  REGION 1..12: note = SnoopTag
KLGDIEFIKVNK

SEQ ID NO: 43 - protein, 116 aa, synthetic construct
  REGION 1..116: note = SpyCatcher
AMVDTLSGLSSEQGQSGDMTIEEDSATHIKFSKRDEDGKELAGATMELRDSSGKTISTWISDGQVKDFYLYPGKYTFVETAAPDGYEVATAITFTVNEQGQVTVNGKATKGDAHID

SEQ ID NO: 44 - protein, 58 aa, synthetic construct
  REGION 1..58: note = Z domain of Protein A
VDNKFNKEQQNAFYEILHLPNLTEEQRNAFIQSLKDDPSVSKEILAEAKKLNDAQAPK

SEQ ID NO: 45 - protein, 56 aa, synthetic construct
  REGION 1..56: note = C2 domain of Protein G
TTYKLVINGKTLKGETTTKAVDAETAEKAFKQYANDNGVDGVWTYDDATKTFTVTE

SEQ ID NO: 46 - protein, 520 aa, Mycoplasma genitalium
  REGION 1..520: note = mature protein M
TNLVNQSGYALVASGRSGNLGFKLFSTQSPSAEVKLKSLSLNDGSYQSEIDLSGGANFREKFRNFANELSEAITNSPKGLDRPVPKTEISGLIKTGDNFITPSFKAGYYDHVASDGSLLSYYQSTEYFNNRVLMPILQTTNGTLMANNRGYDDVFRQVPSFSGWSNTKATTVSTSNNLTYDKWTYFAAKGSPLYDSYPNHFFEDVKTLAIDAKDISALKTTIDSEKPTYLIIRGLSGNGSQLNELQLPESVKKVSLYGDYTGVNVAKQIFANVVELEFYSTSKANSFGFNPLVLGSKTNVIYDLFASKPFTHIDLTQVTLQNSDNSAIDANKLKQAVGDIYNYRRFERQFQGYFAGGYIDKYLVKNVNTNKDSDDDLVYRSLKELNLHLEEAYREGDNTYYRVNENYYPGASIYENERASRDSEFQNEILKRAEQNGVTFDENIKRITASGKYSVQFQKLENDTDSSLERMTKAVEGLVTVIGEEKFETVDITGVSSDTNEVKSLAKELKTNALGVKLKL

SEQ ID NO: 47 - protein, 547 aa, Mycoplasma pneumoniae
  REGION 1..547: note = mature protein M
AVLIVNEVLRLQSGETLIASGRSGNLSFQLYSKVNQNAKSKLNSISLTDGGYRSEIDLGDGSNFREDFRNFANNLSEAITDAPKDLLRPVPKVEVSGLIKTSSTFITPNFKAGYYDQVAADGKTLKYYQSTEYFNNRVVMPILQTTNGTLTANNRAYDDIFVDQGVPKFPGWFHDVDKAYYAGSNGQSEYLFKEWNYYVANGSPLYNVYPNHHFKQIKTIAFDAPRIKQGNTDGINLNLKQRNPDYVIINGLTGDGSTLKDLELPESVKKVSIYGDYHSINVAKQIFKNVLELEFYSTNQDNNFGFNPLVLGDHTNIIYDLFASKPFNYIDLTSLELKDNQDNIDASKLKRAVSDIYIRRRFERQMQGYWAGGYIDRYLVKNTNEKNVNKDNDTVYAALKDINLHLEETYTHGGNTMYRVNENYYPGASAYEAERATRDSEFQKEIVQRAELIGVVFEYGVKNLRPGLKYTVKFESPQEQVALKSTDKFQPVIGSVTDMSKSVTDLIGVLRDNAEILNITNVSKDETVVAELKEKLDRENVFQEIRT

SEQ ID NO: 48 - protein, 14 aa, synthetic construct
  REGION 1..14: note = FcBP-2 immunoglobulin-binding domain
PDCAWHLGELVWCT

SEQ ID NO: 49 - DNA, 13 bp, synthetic construct
  source 1..13: mol_type = other DNA
  misc_feature 1..13: note = stub DNA
  misc_feature 1: note = conjugated to another oligonucleotide through internal amino modifier C6 dT
cggaagagcgtcg

SEQ ID NO: 50 - DNA, 97 bp, synthetic construct
  source 1..97: mol_type = other DNA
  misc_feature 1..97: note = capture DNA
  misc_difference 17..26: note = n is a, c, g, or t
cactcagtccattaacnnnnnnnnnnctagtgtcgcggactacgcattactgagaagcttgctagtcgacgtggtccttttggaccacgtcgactag